European Patent Specification EP 4 396 369 B1, published April 30, 2025. Title: TEMPLATE SWITCH OLIGONUCLEOTIDE (TSO) FOR MRNA 5' ANALYSIS. Applicant: Becton, Dickinson and Company. The sequence listing filed with the application follows.

SEQUENCE LISTING (18 sequences)

SEQ ID NO: 1 - DNA, 20 bp, synthetic construct
  misc_feature 1..20: note = TSO1
  misc_feature 18..20: note = RNA
  source 1..20: mol_type = other DNA
  misc_feature 1..17: note = DNA
tatgcgtagtaggtatgggg

SEQ ID NO: 2 - DNA, 20 bp, synthetic construct
  misc_feature 1..20: note = TSO2
  misc_feature 18..20: note = RNA
  source 1..20: mol_type = other DNA
  misc_feature 1..17: note = DNA
gtggagtcgtgattataggg

SEQ ID NO: 3 - DNA, 30 bp, synthetic construct
  misc_feature 1..30: note = TSO12
  misc_feature 28..30: note = RNA
  source 1..30: mol_type = other DNA
  misc_feature 1..27: note = DNA
tatgcgtagtaggtatggtggagtcgtggg

SEQ ID NO: 4 - DNA, 30 bp, synthetic construct
  misc_feature 1..30: note = TSO21
  misc_feature 28..30: note = RNA
  source 1..30: mol_type = other DNA
  misc_feature 1..27: note = DNA
gtggagtcgttatgcgtagtaggtatgggg

SEQ ID NO: 5 - DNA, 31 bp, synthetic construct
  misc_feature 1..31: note = TSO t21
  misc_feature 29..31: note = RNA
  source 1..31: mol_type = other DNA
  misc_feature 1..28: note = DNA
tgtggagtcgttatgcgtagtaggtatgggg

SEQ ID NO: 6 - DNA, 39 bp, synthetic construct
  misc_feature 1..39: note = TSO t2dT25
  misc_feature 37..39: note = RNA
  source 1..39: mol_type = other DNA
  misc_feature 1..36: note = DNA
tgtggagtcgttttttttttttttttttttttttttggg

SEQ ID NO: 7 - DNA, 30 bp, synthetic construct
  misc_feature 1..30: note = CBO97
  misc_feature 28..30: note = RNA
  source 1..30: mol_type = other DNA
  misc_feature 1..27: note = DNA
aagcagtggtatcaacgcagagtacatggg

SEQ ID NO: 8 - DNA, 21 bp, synthetic construct
  source 1..21: mol_type = other DNA
ttttttttttttttttttttt

SEQ ID NO: 9 - DNA, 20 bp, synthetic construct
  source 1..20: mol_type = other DNA
acaggaaactcatggtgcgt

SEQ ID NO: 10 - DNA, 17 bp, synthetic construct
  source 1..17: mol_type = other DNA
tatgcgtagtaggtatg

SEQ ID NO: 11 - DNA, 20 bp, synthetic construct
  source 1..20: mol_type = other DNA
ccccatacctactacgcata

SEQ ID NO: 12 - DNA, 20 bp, synthetic construct
  source 1..20: mol_type = other DNA
tttttttttttttttttttt

SEQ ID NO: 13 - DNA, 30 bp, synthetic construct
  source 1..30: mol_type = other DNA
ccccatacctactacgcataacgactccac

SEQ ID NO: 14 - DNA, 31 bp, synthetic construct
  source 1..31: mol_type = other DNA
ccccatacctactacgcataacgactccaca

SEQ ID NO: 15 - DNA, 30 bp, synthetic construct
  source 1..30: mol_type = other DNA
cccacgactccaccatacctactacgcata

SEQ ID NO: 16 - DNA, 20 bp, synthetic construct
  source 1..20: mol_type = other DNA
acacgacgctcttccgatct

SEQ ID NO: 17 - DNA, 25 bp, synthetic construct
  source 1..25: mol_type = other DNA
ttttttttttttttttttttttttt

SEQ ID NO: 18 - DNA, 39 bp, synthetic construct
  source 1..39: mol_type = other DNA
cccaaaaaaaaaaaaaaaaaaaaaaaaaacgactccaca